European Patent Application EP 4 810 521 A1, published September 23, 2026. Title: 抗EGFR和HER3双特异性抗体-药物偶联物及其用途. Applicant: 信达生物制药(苏州)有限公司. The sequence listing filed with the application follows.

SEQUENCE LISTING (39 sequences)

SEQ ID NO: 1 - protein, 10 aa, synthetic construct
GFTLSGDWIH

SEQ ID NO: 2 - protein, 17 aa, synthetic construct
EISAAGGYTDYADSVKG

SEQ ID NO: 3 - protein, 12 aa, synthetic construct
ESRVSFEAAMDY

SEQ ID NO: 4 - protein, 11 aa, synthetic construct
RASQNIATDVA

SEQ ID NO: 5 - protein, 7 aa, synthetic construct
SASFLYS

SEQ ID NO: 6 - protein, 9 aa, synthetic construct
QQSEPEPYT

SEQ ID NO: 7 - protein, 121 aa, synthetic construct [sequence omitted]

SEQ ID NO: 8 - protein, 363 aa, synthetic construct
GAAGTGCAACTCGTCGAGAGCGGCGGGGGCCTGGTGCAGCCCGGCGGCTCCCTGAGACTGAGCTGCGCCGCTAGCGGCTTCACCCTGAGCGGCGACTGGATCCACTGGGTGCGGCAAGCCCCTGGCAAGGGCCTCGAGTGGGTCGGGGAAATTAGCGCCGCTGGCGGCTACACCGACTACGCCGACAGCGTGAAGGGCAGATTCACCATCAGCGCCGACACAAGCAAGAACACCGCCTACCTGCAGATGAACAGCCTGAGAGCCGAGGACACCGCCGTGTACTACTGCGCTAGAGAGAGCAGAGTGAGCTTCGAGGCCGCCATGGACTACTGGGGCCAAGGCACCCTGGTGACCGTGAGCAGC

SEQ ID NO: 9 - protein, 107 aa, synthetic construct [sequence omitted]

SEQ ID NO: 10 - protein, 321 aa, synthetic construct
GACATTCAGATGACACAGAGCCCTAGCAGCCTGAGCGCTAGCGTGGGCGACAGAGTGACCATCACCTGCAGAGCTAGCCAAAACATCGCCACCGACGTGGCCTGGTATCAGCAGAAGCCCGGCAAGGCCCCCAAGCTGCTGATCTACAGCGCTAGCTTCCTGTACAGCGGCGTGCCTAGCAGATTCAGCGGCAGCGGCAGCGGCACCGACTTCACCCTGACCATCAGCAGCCTGCAGCCCGAGGACTTCGCCACCTACTACTGTCAGCAGAGCGAGCCCGAGCCCTACACCTTCGGCCAAGGCACCAAGGTGGAGATCAAG

SEQ ID NO: 11 - protein, 330 aa, synthetic construct
ASTKGPSVFPLAPSSKSTSGGTAALGCLVKDYFPEPVTVSWNSGALTSGVHTFPAVLQSSGLYSLSSVVTVPSSSLGTQTYICNVNHKPSNTKVDKKVEPKSCDKTHTCPPCPAPEAAGGPSVFLFPPKPKDTLMISRTPEVTCVVVDVSHEDPEVKFNWYVDGVEVHNAKTKPREEQYNSTYRVVSVLTVLHQDWLNGKEYKCKVSNKALPAPIEKTISKAKGQPREPQVYTLPPSREEMTKNQVSLTCLVKGFYPSDIAVEWESNGQPENNYKTTPPVLDSDGSFFLYSKLTVDKSRWQQGNVFSCSVMHEALHNHYTQKSLSLSPGK

SEQ ID NO: 12 - protein, 451 aa, synthetic construct
EVQLVESGGGLVQPGGSLRLSCAASGFTLSGDWIHWVRQAPGKGLEWVGEISAAGGYTDYADSVKGRFTISADTSKNTAYLQMNSLRAEDTAVYYCARESRVSFEAAMDYWGQGTLVTVSSASTKGPSVFPLAPSSKSTSGGTAALGCLVKDYFPEPVTVSWNSGALTSGVHTFPAVLQSSGLYSLSSVVTVPSSSLGTQTYICNVNHKPSNTKVDKKVEPKSCDKTHTCPPCPAPEAAGGPSVFLFPPKPKDTLMISRTPEVTCVVVDVSHEDPEVKFNWYVDGVEVHNAKTKPREEQYNSTYRVVSVLTVLHQDWLNGKEYKCKVSNKALPAPIEKTISKAKGQPREPQVYTLPPSREEMTKNQVSLTCLVKGFYPSDIAVEWESNGQPENNYKTTPPVLDSDGSFFLYSKLTVDKSRWQQGNVFSCSVMHEALHNHYTQKSLSLSPGK

SEQ ID NO: 13 - protein, 106 aa, synthetic construct
GQPKAAPSVTLFPPSSEELQANKATLVCLISDFYPGAVTVAWKADSSPVKAGVCTTTPSCQSNNKYAASSYLSLTPEQWKSHRSYSCQVTHEGSTVEKTVAPTECS

SEQ ID NO: 14 - protein, 213 aa, synthetic construct
DIQMTQSPSSLSASVGDRVTITCRASQNIATDVAWYQQKPGKAPKLLIYSASFLYSGVPSRFSGSGSGTDFTLTISSLQPEDFATYYCQQSEPEPYTFGQGTKVEIKGQPKAAPSVTLFPPSSEELQANKATLVCLISDFYPGAVTVAWKADSSPVKAGVCTTTPSCQSNNKYAASSYLSLTPEQWKSHRSYSCQVTHEGSTVEKTVAPTECS

SEQ ID NO: 15 - protein, 330 aa, synthetic construct
CSTKGPSVFPLAPSSKSTSGGTAALGCLVKDYFPEPVTVSWNSGALTSGVHTFPAVLQSSGLYSLSSVVTVPSSSLGTQTYICNVNHKPSNTKVDKKVEPKSCDKTHTCPPCPAPEAAGGPCVFLFPPKPKDTLMISRTPEVTCVVVDVSHEDPEVKFNWYVDGVEVHNAKTKPREEQYNSTYRVVSVLTVLHQDWLNGKEYKCKVSNKALPAPIEKTISKAKGQPREPQVYTLPPSREEMTKNQVSLTCLVKGFYPSDIAVEWESNGQPENNYKTTPPVLDSDGSFFLYSKLTVDKSRWQQGNVFSCSVMHEALHNHYTQKSLSLSPGK

SEQ ID NO: 16 - protein, 451 aa, synthetic construct
EVQLVESGGGLVQPGGSLRLSCAASGFTLSGDWIHWVRQAPGKGLEWVGEISAAGGYTDYADSVKGRFTISADTSKNTAYLQMNSLRAEDTAVYYCARESRVSFEAAMDYWGQGTLVTVSSCSTKGPSVFPLAPSSKSTSGGTAALGCLVKDYFPEPVTVSWNSGALTSGVHTFPAVLQSSGLYSLSSVVTVPSSSLGTQTYICNVNHKPSNTKVDKKVEPKSCDKTHTCPPCPAPEAAGGPCVFLFPPKPKDTLMISRTPEVTCVVVDVSHEDPEVKFNWYVDGVEVHNAKTKPREEQYNSTYRVVSVLTVLHQDWLNGKEYKCKVSNKALPAPIEKTISKAKGQPREPQVYTLPPSREEMTKNQVSLTCLVKGFYPSDIAVEWESNGQPENNYKTTPPVLDSDGSFFLYSKLTVDKSRWQQGNVFSCSVMHEALHNHYTQKSLSLSPGK

SEQ ID NO: 17 - protein, 107 aa, synthetic construct [sequence omitted]

SEQ ID NO: 18 - protein, 214 aa, synthetic construct
DIQMTQSPSSLSASVGDRVTITCRASQNIATDVAWYQQKPGKAPKLLIYSASFLYSGVPSRFSGSGSGTDFTLTISSLQPEDFATYYCQQSEPEPYTFGQGTKVEIKRTVAAPSVFIFPPSDEQLKSGTASVVCLLNNFYPREAKVQWKVDNALQSGNSQESVTEQDSKDSTYSLSSTLTLSKADYEKHKVYACEVTHQGLSSPVTKSFNRGEC

SEQ ID NO: 19 - protein, 330 aa, synthetic construct
CSTKGPSVFPLAPSSKSTSGGTAALGCLVKDYFPEPVTVSWNSGALTSGVHTFPAVLQSSGLYSLSSVVTVPSSSLGTQTYICNVNHKPSNTKVDKKVEPKSCDKTHTCPPCPAPEAAGGPSVFLFPPKPKDTLMISRTPEVTCVVVDVSHEDPEVKFNWYVDGVEVHNAKTKPREEQYNSTYRVVSVLTVLHQDWLNGKEYKCKVSNKALPAPIEKTISKAKGQPREPQVYTLPPSREEMTKNQVSLTCLVKGFYPSDIAVEWESNGQPENNYKTTPPVLDSDGSFFLYSKLTVDKSRWQQGNVFSCSVMHEALHNHYTQKSLSLSPGK

SEQ ID NO: 20 - protein, 451 aa, synthetic construct
EVQLVESGGGLVQPGGSLRLSCAASGFTLSGDWIHWVRQAPGKGLEWVGEISAAGGYTDYADSVKGRFTISADTSKNTAYLQMNSLRAEDTAVYYCARESRVSFEAAMDYWGQGTLVTVSSCSTKGPSVFPLAPSSKSTSGGTAALGCLVKDYFPEPVTVSWNSGALTSGVHTFPAVLQSSGLYSLSSVVTVPSSSLGTQTYICNVNHKPSNTKVDKKVEPKSCDKTHTCPPCPAPEAAGGPSVFLFPPKPKDTLMISRTPEVTCVVVDVSHEDPEVKFNWYVDGVEVHNAKTKPREEQYNSTYRVVSVLTVLHQDWLNGKEYKCKVSNKALPAPIEKTISKAKGQPREPQVYTLPPSREEMTKNQVSLTCLVKGFYPSDIAVEWESNGQPENNYKTTPPVLDSDGSFFLYSKLTVDKSRWQQGNVFSCSVMHEALHNHYTQKSLSLSPGK

SEQ ID NO: 21 - protein, 106 aa, synthetic construct
GQPKAAPSVTLFPPSSEELQANKATLVCLISDFYPGAVTVAWKADSSPVKAGVCTTTPSKQSNNKYAASSYLSLTPEQWKSHRSYSCQVTHEGSTVEKTVAPTECS

SEQ ID NO: 22 - protein, 213 aa, synthetic construct
DIQMTQSPSSLSASVGDRVTITCRASQNIATDVAWYQQKPGKAPKLLIYSASFLYSGVPSRFSGSGSGTDFTLTISSLQPEDFATYYCQQSEPEPYTFGQGTKVEIKGQPKAAPSVTLFPPSSEELQANKATLVCLISDFYPGAVTVAWKADSSPVKAGVCTTTPSKQSNNKYAASSYLSLTPEQWKSHRSYSCQVTHEGSTVEKTVAPTECS

SEQ ID NO: 23 - protein, 330 aa, synthetic construct
ASTKGPSVFPLAPSSKSTSGGTAALGCLVKDYFPEPVTVSWNSGALTSGVHTFPAVLQSSGLYSLSSVVTVPSSSLGTQTYICNVNHKPSNTKVDKKVEPKSCDKTHTCPPCPAPEAAGGPCVFLFPPKPKDTLMISRTPEVTCVVVDVSHEDPEVKFNWYVDGVEVHNAKTKPREEQYNSTYRVVSVLTVLHQDWLNGKEYKCKVSNKALPAPIEKTISKAKGQPREPQVYTLPPSREEMTKNQVSLTCLVKGFYPSDIAVEWESNGQPENNYKTTPPVLDSDGSFFLYSKLTVDKSRWQQGNVFSCSVMHEALHNHYTQKSLSLSPGK

SEQ ID NO: 24 - protein, 451 aa, synthetic construct
EVQLVESGGGLVQPGGSLRLSCAASGFTLSGDWIHWVRQAPGKGLEWVGEISAAGGYTDYADSVKGRFTISADTSKNTAYLQMNSLRAEDTAVYYCARESRVSFEAAMDYWGQGTLVTVSSASTKGPSVFPLAPSSKSTSGGTAALGCLVKDYFPEPVTVSWNSGALTSGVHTFPAVLQSSGLYSLSSVVTVPSSSLGTQTYICNVNHKPSNTKVDKKVEPKSCDKTHTCPPCPAPEAAGGPCVFLFPPKPKDTLMISRTPEVTCVVVDVSHEDPEVKFNWYVDGVEVHNAKTKPREEQYNSTYRVVSVLTVLHQDWLNGKEYKCKVSNKALPAPIEKTISKAKGQPREPQVYTLPPSREEMTKNQVSLTCLVKGFYPSDIAVEWESNGQPENNYKTTPPVLDSDGSFFLYSKLTVDKSRWQQGNVFSCSVMHEALHNHYTQKSLSLSPGK

SEQ ID NO: 25 - protein, 106 aa, synthetic construct
GQPKAAPSVTLFPPSSEELQANKATLVCLISDFYPGAVTVAWKADSSPVKAGVETTTPSCQSNNKYAASSYLSLTPEQWKSHRSYSCQVTHEGSTVEKTVAPTECS

SEQ ID NO: 26 - protein, 213 aa, synthetic construct
DIQMTQSPSSLSASVGDRVTITCRASQNIATDVAWYQQKPGKAPKLLIYSASFLYSGVPSRFSGSGSGTDFTLTISSLQPEDFATYYCQQSEPEPYTFGQGTKVEIKGQPKAAPSVTLFPPSSEELQANKATLVCLISDFYPGAVTVAWKADSSPVKAGVETTTPSCQSNNKYAASSYLSLTPEQWKSHRSYSCQVTHEGSTVEKTVAPTECS

SEQ ID NO: 27 - protein, 702 aa, synthetic construct
QVQLKQSGPGLVQPSQSLSITCTVSGFSLTNYGVHWVRQSPGKGLEWLGVIWSGGNTDYNTPFTSRLSINKDNSKSQVFFKMNSLQSNDTAIYYCARALTYYDYEFAYWGQGTLVTVSSASTKGPSVFPLAPSSKSTSGGTAALGCLVKDYFPEPVTVSWNSGALTSGVHTFPAVLQSSGLYSLSSVVTVPSSSLGTQTYICNVNHKPSNTKVDKKVEPKSCDKTHTCPPCPAPELLGGPSVFLFPPKPKDTLMISRTPEVTCVVVDVSHEDPEVKFNWYVDGVEVHNAKTKPREEQYNSTYRVVSVLTVLHQDWLNGKEYKCKVSNKALPAPIEKTISKAKGQPREPQVYTLPPSRDELTKNQVSLTCLVKGFYPSDIAVEWESNGQPENNYKTTPPVLDSDGSFFLYSKLTVDKSRWQQGNVFSCSVMHEALHNHYTQKSLSLSPGGGGGSGGGGSQVQLQESGGGLVKPGGSLRLSCAASGFTFSSYWMSWVRQAPGKGLEWVANINRDGSASYYVDSVKGRFTISRDDAKNSLYLQMNSLRAEDTAVYYCARDRGVGYFDLWGRGTLVTVSSGGGGSGGGGSGGGGSQSALTQPASVSGSPGQSITISCTGTSSDVGGYNFVSWYQQHPGKAPKLMIYDVSDRPSGVSDRFSGSKSGNTASLIISGLQADDEADYYCSSYGSSSTHVIFGGGTKVTVL

SEQ ID NO: 28 - protein, 214 aa, synthetic construct
DILLTQSPVILSVSPGERVSFSCRASQSIGTNIHWYQQRTNGSPRLLIKYASESISGIPSRFSGSGSGTDFTLSINSVESEDIADYYCQQNNNWPTTFGAGTKLELKRTVAAPSVFIFPPSDEQLKSGTASVVCLLNNFYPREAKVQWKVDNALQSGNSQESVTEQDSKDSTYSLSSTLTLSKADYEKHKVYACEVTHQGLSSPVTKSFNRGEC

SEQ ID NO: 29 - protein, 451 aa, synthetic construct
EVQLVESGGGLVQPGGSLRLSCAASGFTLSGDWIHWVRQAPGKGLEWVGEISAAGGYTDYADSVKGRFTISADTSKNTAYLQMNSLRAEDTAVYYCARESRVSFEAAMDYWGQGTLVTVSSASTKGPSVFPLAPSSKSTSGGTAALGCLVKDYFPEPVTVSWNSGALTSGVHTFPAVLQSSGLYSLSSVVTVPSSSLGTQTYICNVNHKPSNTKVDKKVEPKSCDKTHTCPPCPAPELLGGPSVFLFPPKPKDTLMISRTPEVTCVVVDVSHEDPEVKFNWYVDGVEVHNAKTKPREEQYNSTYRVVSVLTVLHQDWLNGKEYKCKVSNKALPAPIEKTISKAKGQPREPQVYTLPPSRDELTKNQVSLTCLVKGFYPSDIAVEWESNGQPENNYKTTPPVLDSDGSFFLYSKLTVDKSRWQQGNVFSCSVMHEALHNHYTQKSLSLSPGK

SEQ ID NO: 30 - protein, 214 aa, synthetic construct; identical to SEQ ID NO: 18

SEQ ID NO: 31 - protein, 456 aa, synthetic construct
QVQLVQSGAEVKKPGASVKVSCQASGYRFSNFVIHWVRQAPGQRFEWMGWINPYNGNKEFSAKFQDRVTFTADTSANTAYMELRSLRSADTAVYYCARVGPYSWDDSPQDNYYMDVWGKGTTVIVSSASTKGPSVFPLAPSSKSTSGGTAALGCLVKDYFPEPVTVSWNSGALTSGVHTFPAVLQSSGLYSLSSVVTVPSSSLGTQTYICNVNHKPSNTKVDKKVEPKSCDKTHTCPPCPAPEAAGGPSVFLFPPKPKDTLMISRTPEVTCVVVDVSHEDPEVKFNWYVDGVEVHNAKTKPREEQYNSTYRVVSVLTVLHQDWLNGKEYKCKVSNKALPAPIEKTISKAKGQPREPQVYTLPPSRDELTKNQVSLTCLVKGFYPSDIAVEWESNGQPENNYKTTPPVLDSDGSFFLYSKLTVDKSRWQQGNVFSCSVMHEALHNHYTQKSLSLSPG

SEQ ID NO: 32 - protein, 215 aa, synthetic construct
EIVLTQSPGTLSLSPGERATFSCRSSHSIRSRRVAWYQHKPGQAPRLVIHGVSNRASGISDRFSGSGSGTDFTLTITRVEPEDFALYYCQVYGASSYTFGQGTKLERKRTVAAPSVFIFPPSDEQLKSGTASVVCLLNNFYPREAKVQWKVDNALQSGNSQESVTEQDSKDSTYSLSSTLTLSKADYEKHKVYACEVTHQGLSSPVTKSFNRGEC

SEQ ID NO: 33 - protein, 447 aa, synthetic construct
QVQLQQWGAGLLKPSETLSLTCAVYGGSFSGYYWSWIRQPPGKGLEWIGEINHSGSTNYNPSLKSRVTISVETSKNQFSLKLSSVTAADTAVYYCARDKWTWYFDLWGRGTLVTVSSASTKGPSVFPLAPSSKSTSGGTAALGCLVKDYFPEPVTVSWNSGALTSGVHTFPAVLQSSGLYSLSSVVTVPSSSLGTQTYICNVNHKPSNTKVDKRVEPKSCDKTHTCPPCPAPELLGGPSVFLFPPKPKDTLMISRTPEVTCVVVDVSHEDPEVKFNWYVDGVEVHNAKTKPREEQYNSTYRVVSVLTVLHQDWLNGKEYKCKVSNKALPAPIEKTISKAKGQPREPQVYTLPPSREEMTKNQVSLTCLVKGFYPSDIAVEWESNGQPENNYKTTPPVLDSDGSFFLYSKLTVDKSRWQQGNVFSCSVMHEALHNHYTQKSLSLSPGK

SEQ ID NO: 34 - protein, 220 aa, synthetic construct
DIEMTQSPDSLAVSLGERATINCRSSQSVLYSSSNRNYLAWYQQNPGQPPKLLIYWASTRESGVPDRFSGSGSGTDFTLTISSLQAEDVAVYYCQQYYSTPRTFGQGTKVEIKRTVAAPSVFIFPPSDEQLKSGTASVVCLLNNFYPREAKVQWKVDNALQSGNSQESVTEQDSKDSTYSLSSTLTLSKADYEKHKVYACEVTHQGLSSPVTKSFNRGEC

SEQ ID NO: 35 - protein, 330 aa, synthetic construct
ASTKGPSVFPLAPSSKSTSGGTAALGCLVKDYFPEPVTVSWNSGALTSGVHTFPAVLQSSGLYSLSSVVTVPSSSLGTQTYICNVNHKPSNTKVDKKVEPKSCDKTHTCPPCPAPELLGGPSVFLFPPKPKDTLMISRTPEVTCVVVDVSHEDPEVKFNWYVDGVEVHNAKTKPREEQYNSTYRVVSVLTVLHQDWLNGKEYKCKVSNKALPAPIEKTISKAKGQPREPQVYTLPPSREEMTKNQVSLTCLVKGFYPSDIAVEWESNGQPENNYKTTPPVLDSDGSFFLYSKLTVDKSRWQQGNVFSCSVMHEALHNHYTQKSLSLSPGK

SEQ ID NO: 36 - protein, 106 aa, synthetic construct
GQPKAAPSVTLFPPSSEELQANKATLVCLISDFYPGAVTVAWKADSSPVKAGVETTTPSKQSNNKYAASSYLSLTPEQWKSHRSYSCQVTHEGSTVEKTVAPTECS

SEQ ID NO: 37 - skipped

SEQ ID NO: 38 - protein, 449 aa, synthetic construct
QVQLKQSGPGLVQPSQSLSITCTVSGFSLTNYGVHWVRQSPGKGLEWLGVIWSGGNTDYNTPFTSRLSINKDNSKSQVFFKMNSLQSNDTAIYYCARALTYYDYEFAYWGQGTLVTVSAASTKGPSVFPLAPSSKSTSGGTAALGCLVKDYFPEPVTVSWNSGALTSGVHTFPAVLQSSGLYSLSSVVTVPSSSLGTQTYICNVNHKPSNTKVDKKVEPKSCDKTHTCPPCPAPELLGGPSVFLFPPKPKDTLMISRTPEVTCVVVDVSHEDPEVKFNWYVDGVEVHNAKTKPREEQYNSTYRVVSVLTVLHQDWLNGKEYKCKVSNKALPAPIEKTISKAKGQPREPQVYTLPPSRDELTKNQVSLTCLVKGFYPSDIAVEWESNGQPENNYKTTPPVLDSDGSFFLYSKLTVDKSRWQQGNVFSCSVMHEALHNHYTQKSLSLSPGK

SEQ ID NO: 39 - protein, 214 aa, synthetic construct; identical to SEQ ID NO: 28